European Patent Application EP 4 163 376 A1, published April 12, 2023. Title: INSULIN ASPART DERIVATIVE, AND PREPARATION METHOD THEREFOR AND USE THEREOF. Applicant: NINGBO KUNPENG BIOTECH CO., LTD. The sequence listing filed with the application follows.

SEQUENCE LISTING (25 sequences)

SEQ ID NO: 1 - protein, 88 aa, Artificial Sequence
  Insulin aspart fusion protein
GIKANFKIRHNVEDVQLADHYQQNTPIGENLYFQGRFVNQHLCGSHLVEALYLVCGERGFFYTDKTRGIVEQCCTSICSLYQLENYCN

SEQ ID NO: 2 - protein, 12 aa, Artificial Sequence
  Leader peptide
MVSKGEELFTGV

SEQ ID NO: 3 - protein, 28 aa, Artificial Sequence
  Green fluorescent protein folding unit
GIKANFKIRHNVEDVQLADHYQQNTPIG

SEQ ID NO: 4 - protein, 7 aa, Artificial Sequence
  Restriction site of TEV enzyme
ENLYFQG

SEQ ID NO: 5 - protein, 52 aa, Artificial Sequence
  Insulin aspart
FVNQHLCGSHLVEALYLVCGERGFFYTDKTRGIVEQCCTSICSLYQLENYCN

SEQ ID NO: 6 - protein, 6 aa, Artificial Sequence
  Linker peptide
RRGSKR

SEQ ID NO: 7 - protein, 6 aa, Artificial Sequence
  Linker peptide
RRAAKR

SEQ ID NO: 8 - protein, 9 aa, Artificial Sequence
  Linker peptide
RRYPGDVKR

SEQ ID NO: 9 - protein, 35 aa, Artificial Sequence
  Linker peptide
RREAEDLQVGQVELGGGPGAGSLQPLALEGSLQKR

SEQ ID NO: 10 - protein, 104 aa, Artificial Sequence
  Fusion protein
MKKLLFAIPLVVPFYSHSTMELEICSWYHMGIRSFLEQKLISEEDLNSAVDRFVNQHLCGSHLVEALYLVCGERGFFYTDKTRGIVEQCCTSICSLYQLENYCN

SEQ ID NO: 11 - protein, 13 aa, Artificial Sequence
  β-folding unit
VPILVELDGDVNG

SEQ ID NO: 12 - protein, 14 aa, Artificial Sequence
  β-folding unit
HKFSVRGEGEGDAT

SEQ ID NO: 13 - protein, 10 aa, Artificial Sequence
  β-folding unit
KLTLKFICTT

SEQ ID NO: 14 - protein, 11 aa, Artificial Sequence
  β-folding unit
YVQERTISFKD

SEQ ID NO: 15 - protein, 13 aa, Artificial Sequence
  β-folding unit
TYKTRAEVKFEGD

SEQ ID NO: 16 - protein, 13 aa, Artificial Sequence
  β-folding unit
TLVNRIELKGIDF

SEQ ID NO: 17 - protein, 10 aa, Artificial Sequence
  β-folding unit
HNVYITADKQ

SEQ ID NO: 18 - protein, 14 aa, Artificial Sequence
  β-folding unit
GIKANFKIRHNVED

SEQ ID NO: 19 - protein, 14 aa, Artificial Sequence
  β-folding unit
VQLADHYQQNTPIG

SEQ ID NO: 20 - protein, 12 aa, Artificial Sequence
  β-folding unit
HYLSTQSVLSKD

SEQ ID NO: 21 - protein, 13 aa, Artificial Sequence
  β-folding unit
HMVLLEFVTAAGI

SEQ ID NO: 22 - protein, 99 aa, Artificial Sequence
  Fusion protein
VQLADHYQQNTPIGHYLSTQSVLSKDHMVLLEFVTAAGIENLYFQGRFVNQHLCGSHLVEALYLVCGERGFFYTDKTRGIVEQCCTSICSLYQLENYCN

SEQ ID NO: 23 - protein, 85 aa, Artificial Sequence
  Fusion protein
HYLSTQSVLSKDHMVLLEFVTAAGIENLYFQGRFVNQHLCGSHLVEALYLVCGERGFFYTDKTRGIVEQCCTSICSLYQLENYCN

SEQ ID NO: 24 - protein, 39 aa, Artificial Sequence
  Green fluorescent protein folding unit
VQLADHYQQNTPIGHYLSTQSVLSKDHMVLLEFVTAAGI

SEQ ID NO: 25 - protein, 25 aa, Artificial Sequence
  Green fluorescent protein folding unit
HYLSTQSVLSKDHMVLLEFVTAAGI